European Patent Application EP 4 420 666 A1, published August 28, 2024. Title: 抗がん免疫増強作用又は／及び免疫チェックポイント阻害増強作用を有する医薬組成物. Applicant: 国立大学法人九州大学. The sequence listing filed with the application follows.

SEQUENCE LISTING (9 sequences)

SEQ ID NO: 1 - protein, 17 aa, synthetic construct
  source 1..17: note = Amino acid sequence of OVA peptide (OVA323-339)
ISQAVHAAHAEINEAGR

SEQ ID NO: 2 - DNA, 24 bp, synthetic construct
  source 1..24: mol_type = other DNA
caccgatcttgtagcgtcgcagga

SEQ ID NO: 3 - DNA, 24 bp, synthetic construct
  source 1..24: mol_type = other DNA
aaactcctgcgacgctacaagatc

SEQ ID NO: 4 - DNA, 33 bp, synthetic construct
  source 1..33: mol_type = other DNA
accggtacctgtgaggttagagcccagttccag

SEQ ID NO: 5 - DNA, 30 bp, synthetic construct
  source 1..30: mol_type = other DNA
accgcggccgcacccggacttctcgccttc

SEQ ID NO: 6 - DNA, 31 bp, synthetic construct
  source 1..31: mol_type = other DNA
tccggatcctggggacccagggatacaggac

SEQ ID NO: 7 - DNA, 32 bp, synthetic construct
  source 1..32: mol_type = other DNA
gacgtcgaccagtgtctgaaagggtatccagg

SEQ ID NO: 8 - DNA, 20 bp, synthetic construct
  source 1..20: mol_type = other DNA
tgtgtccgtcgtggatctga

SEQ ID NO: 9 - DNA, 21 bp, synthetic construct
  source 1..21: mol_type = other DNA
ttgctgttgaagtcgcaggag